European Patent Application EP 4 725 301 A1, published April 15, 2026. Title: SESAME WITH IMPROVED TASTE FROM SHATTER RESISTANT SESAME PLANTS. Applicant: EQUI-NOM LTD. The sequence listing filed with the application follows.

SEQUENCE LISTING (24 sequences)

SEQ ID NO: 1 - DNA, 122 bp, Sesamum indicum
  misc_feature 1..122: note = Description of sequence: sequence containing signle nucelotide polymorphism
  source 1..122: mol_type = other DNA
  misc_feature 61: note = Single nucleotide polymorphism base
aacctctagaagtatcttttgaaagaatccattcaatacctttccttcattggcttggttaccaatctcctcattctcttcctgcagggtcctgcattttgccattaacatctttcccattt

SEQ ID NO: 2 - DNA, 122 bp, Sesamum indicum
  misc_feature 1..122: note = Description of sequence: sequence containing signle nucelotide polymorphism
  source 1..122: mol_type = other DNA
  misc_feature 61: note = Single nucleotide polymorphism base
aacctctagaagtatcttttgaaagaatccattcaatacctttccttcattggcttggttgccaatctcctcattctcttcctgcagggtcctgcattttgccattaacatctttcccattt

SEQ ID NO: 3 - DNA, 201 bp, Sesamum indicum
  misc_feature 1..201: note = Description of sequence: sequence containing signle nucelotide polymorphism
  source 1..201: mol_type = other DNA
  misc_feature 101: note = Single nucleotide polymorphism base
tacacacaactcacttttgtatctcaatactcacattcatattcttcttactacatacttttgggcaacttgataaggtctagttctctaatcatcttgtaacgtgctcacaatagaaaacgctggttgaggcttttttggttttatcttggggtagttgtgagccgatagtacctgcaaggagggaggtcattacgattt

SEQ ID NO: 4 - DNA, 201 bp, Sesamum indicum
  misc_feature 1..201: note = Description of sequence: sequence containing signle nucelotide polymorphism
  source 1..201: mol_type = other DNA
  misc_feature 101: note = Single nucleotide polymorphism base
tacacacaactcacttttgtatctcaatactcacattcatattcttcttactacatacttttgggcaacttgataaggtctagttctctaatcatcttgtgacgtgctcacaatagaaaacgctggttgaggcttttttggttttatcttggggtagttgtgagccgatagtacctgcaaggagggaggtcattacgattt

SEQ ID NO: 5 - DNA, 201 bp, Sesamum indicum
  misc_feature 1..201: note = Description of sequence: sequence containing signle nucelotide polymorphism
  source 1..201: mol_type = other DNA
  misc_feature 101: note = Single nucleotide polymorphism base
atttatagggctaaatgtgccccaccttccggtccacgtggtgtcatctcaaatcataagttgttagatgatctacggtctagggtcatcagagcgggtcaggtcgagcgattctacttgagagagaaagtgttggaatgggtgaccaaaaagtcaattggagtgattatttgccattcgtcaatctttattaaataatat

SEQ ID NO: 6 - DNA, 201 bp, Sesamum indicum
  misc_feature 1..201: note = Description of sequence: sequence containing signle nucelotide polymorphism
  source 1..201: mol_type = other DNA
  misc_feature 101: note = Single nucleotide polymorphism base
atttatagggctaaatgtgccccaccttccggtccacgtggtgtcatctcaaatcataagttgttagatgatctacggtctagggtcatcagagcgggtcgggtcgagcgattctacttgagagagaaagtgttggaatgggtgaccaaaaagtcaattggagtgattatttgccattcgtcaatctttattaaataatat

SEQ ID NO: 7 - DNA, 201 bp, Sesamum indicum
  misc_feature 1..201: note = Description of sequence: sequence containing signle nucelotide polymorphism
  source 1..201: mol_type = other DNA
  misc_feature 101: note = Single nucleotide polymorphism base
ggtgtattttacaattttatgctgctttatgcttaagtgtcgtggaactcgcaaagtttggctccgccacgaaattttgtactatcgagattgttataagatattgctgagaaagatcaaatcatgagaagactgaacaaaaagattttatttctggatcaaattctggagtggagaagaggaaagcagtgagtgtgaaaa

SEQ ID NO: 8 - DNA, 201 bp, Sesamum indicum
  misc_feature 1..201: note = Description of sequence: sequence containing signle nucelotide polymorphism
  source 1..201: mol_type = other DNA
  misc_feature 101: note = Single nucleotide polymorphism base
ggtgtattttacaattttatgctgctttatgcttaagtgtcgtggaactcgcaaagtttggctccgccacgaaattttgtactatcgagattgttataaggtattgctgagaaagatcaaatcatgagaagactgaacaaaaagattttatttctggatcaaattctggagtggagaagaggaaagcagtgagtgtgaaaa

SEQ ID NO: 9 - DNA, 201 bp, Sesamum indicum
  misc_feature 1..201: note = Description of sequence: sequence containing signle nucelotide polymorphism
  source 1..201: mol_type = other DNA
  misc_feature 101: note = Single nucleotide polymorphism base
cttttgttattttacttattaaaaatttaaaaaataaataagaagtgtaattattattgtttcatttttaccaaaaagttcggtttaccgaataccgattcgaaattcctaaacagattaggtagtatctgttcggtattctggttcatttggattttacctaacatctgtaacaactcttttggccttggtggttccaat

SEQ ID NO: 10 - DNA, 201 bp, Sesamum indicum
  misc_feature 1..201: note = Description of sequence: sequence containing signle nucelotide polymorphism
  source 1..201: mol_type = other DNA
  misc_feature 101: note = Single nucleotide polymorphism base
cttttgttattttacttattaaaaatttaaaaaataaataagaagtgtaattattattgtttcatttttaccaaaaagttcggtttaccgaataccgatttgaaattcctaaacagattaggtagtatctgttcggtattctggttcatttggattttacctaacatctgtaacaactcttttggccttggtggttccaat

SEQ ID NO: 11 - DNA, 160 bp, Sesamum indicum
  misc_feature 1..160: note = Description of sequence: sequence containing signle nucelotide polymorphism
  source 1..160: mol_type = other DNA
  misc_feature 101: note = Single nucleotide polymorphism base
aaaaacaagatcatgcttaattctatggtcgattatgtatgcaaagacgacaatcattcatgatagataaattggttataaccattagtacgacctaacaaccttacctttggacagtcaaggaacgtcgattaactaaatccctaatcagtaaataatc

SEQ ID NO: 12 - DNA, 160 bp, Sesamum indicum
  misc_feature 1..160: note = Description of sequence: sequence containing signle nucelotide polymorphism
  source 1..160: mol_type = other DNA
  misc_feature 101: note = Single nucleotide polymorphism base
aaaaacaagatcatgcttaattctatggtcgattatgtatgcaaagacgacaatcattcatgatagataaattggttatgaccattagtacgacctaacaaccttacctttggacagtcaaggaacgtcgattaactaaatccctaatcagtaaataatc

SEQ ID NO: 13 - DNA, 201 bp, Sesamum indicum
  misc_feature 1..201: note = Description of sequence: sequence containing signle nucelotide polymorphism
  source 1..201: mol_type = other DNA
  misc_feature 101: note = Single nucleotide polymorphism base
gcgtaaaagcatgacttacgttaaaagctactactaaagtaaaatccccaatagagtattctgtctcatctcaacccatcgactttcccatcctcaacatttccatcattctttccgccctttaagctatggaaggaactaactactcctgcttaattcctaacctcatctcaaaacacactacctgcgacttgtaatgtt

SEQ ID NO: 14 - DNA, 201 bp, Sesamum indicum
  misc_feature 1..201: note = Description of sequence: sequence containing signle nucelotide polymorphism
  source 1..201: mol_type = other DNA
  misc_feature 101: note = Single nucleotide polymorphism base
gcgtaaaagcatgacttacgttaaaagctactactaaagtaaaatccccaatagagtattctgtctcatctcaacccatcgactttcccatcctcaacatctccatcattctttccgccctttaagctatggaaggaactaactactcctgcttaattcctaacctcatctcaaaacacactacctgcgacttgtaatgtt

SEQ ID NO: 15 - DNA, 201 bp, Sesamum indicum
  misc_feature 1..201: note = Description of sequence: sequence containing signle nucelotide polymorphism
  source 1..201: mol_type = other DNA
  misc_feature 101: note = Single nucleotide polymorphism base
ttttgtttgataggaggaaaagatggattcaagtttaggctgtgcatcacgctgtattccctattagatcactggctgaccatgcaaggacatccatgttctcatgcaggaaggtagtgaattctcctattatttcaaggaatagttgggagccgatccgcctctcttgatacaagctggaggcaccgtacctcttgaatg

SEQ ID NO: 16 - DNA, 201 bp, Sesamum indicum
  misc_feature 1..201: note = Description of sequence: sequence containing signle nucelotide polymorphism
  source 1..201: mol_type = other DNA
  misc_feature 101: note = Single nucleotide polymorphism base
ttttgtttgataggaggaaaagatggattcaagtttaggctgtgcatcacgctgtattccctattagatcactggctgaccatgcaaggacatccatgttttcatgcaggaaggtagtgaattctcctattatttcaaggaatagttgggagccgatccgcctctcttgatacaagctggaggcaccgtacctcttgaatg

SEQ ID NO: 17 - DNA, 201 bp, Sesamum indicum
  misc_feature 1..201: note = Description of sequence: sequence containing signle nucelotide polymorphism
  source 1..201: mol_type = other DNA
  misc_feature 101: note = Single nucleotide polymorphism base
ccgaaagtagtgaagtccagcctactttcggtcccggtgggctcataagtcgataaatatcgtgggtcgtgggcttcccactagtacacctccatacaatgcggtcgtcacccccgtaaatcctttgcaaggtatgtataatctccatgtactccatatccgtaatcaatggccaatgccattgtccctcatgaataatgg

SEQ ID NO: 18 - DNA, 201 bp, Sesamum indicum
  misc_feature 1..201: note = Description of sequence: sequence containing signle nucelotide polymorphism
  source 1..201: mol_type = other DNA
  misc_feature 101: note = Single nucleotide polymorphism base
ccgaaagtagtgaagtccagcctactttcggtcccggtgggctcataagtcgataaatatcgtgggtcgtgggcttcccactagtacacctccatacaatacggtcgtcacccccgtaaatcctttgcaaggtatgtataatctccatgtactccatatccgtaatcaatggccaatgccattgtccctcatgaataatgg

SEQ ID NO: 19 - DNA, 122 bp, Sesamum indicum
  misc_feature 1..122: note = Description of sequence: sequence containing signle nucelotide polymorphism
  source 1..122: mol_type = other DNA
  misc_feature 61: note = Single nucleotide polymorphism base
agaaaaataagtaaaggtatatgctcgaatgcagcaacgagagaaatcctggtttgcatgttctcctaaatcaaggctgcagtatatggcgcccacgccaagactcccttccctgagcgaac

SEQ ID NO: 20 - DNA, 122 bp, Sesamum indicum
  misc_feature 1..122: note = Description of sequence: sequence containing signle nucelotide polymorphism
  source 1..122: mol_type = other DNA
  misc_feature 61: note = Single nucleotide polymorphism base
agaaaaataagtaaaggtatatgctcgaatgcagcaacgagagaaatcctggtttgcatgctctcctaaatcaaggctgcagtatatggcgcccacgccaagactcccttccctgagcgaac

SEQ ID NO: 21 - DNA, 160 bp, Sesamum indicum
  misc_feature 1..160: note = Description of sequence: sequence containing signle nucelotide polymorphism, Loci QTL 11
  source 1..160: mol_type = genomic DNA
  misc_feature 80: note = Single nucleotide polymorphism base
ggagtggtgctcaccagcccaaaagggaacgaactggaatatgctttgcgtttcgactttagcgcttcaaataatgaggctgaatattaagcgcttattggaggtaccaggatggccttgaatacaagagctaaaagtctaattcctactccgattccca

SEQ ID NO: 22 - DNA, 160 bp, Sesamum indicum
  misc_feature 1..160: note = Description of sequence: sequence containing signle nucelotide polymorphism, Loci QTL 11
  source 1..160: mol_type = genomic DNA
  misc_feature 80: note = Single nucleotide polymorphism base
ggagtggtgctcaccagcccaaaagggaacgaactggaatatgctttgcgtttcgactttagcgcttcaaataatgaggttgaatattaagcgcttattggaggtaccaggatggccttgaatacaagagctaaaagtctaattcctactccgattccca

SEQ ID NO: 23 - DNA, 201 bp, Sesamum indicum
  misc_feature 1..201: note = Description of sequence: sequence containing signle nucelotide polymorphism, Loci QTL 12
  source 1..201: mol_type = genomic DNA
  misc_feature 101: note = Single nucleotide polymorphism base
tctaaaagacaccccaacaactcgctattaaacaaatcaagtatgatatgtgagagtagtgctctaattatacctacctactttacaaacaaatttgaattcccttgaaagaaatgattgcccttttatgccttttgttttgtaatgcctcaggtttaatattaataatacagacactcacccccaagattcatttctcta

SEQ ID NO: 24 - DNA, 201 bp, Sesamum indicum
  misc_feature 1..201: note = Description of sequence: sequence containing signle nucelotide polymorphism, Loci QTL 12
  source 1..201: mol_type = genomic DNA
  misc_feature 101: note = Single nucleotide polymorphism base
tctaaaagacaccccaacaactcgctattaaacaaatcaagtatgatatgtgagagtagtgctctaattatacctacctactttacaaacaaatttgaatccccttgaaagaaatgattgcccttttatgccttttgttttgtaatgcctcaggtttaatattaataatacagacactcacccccaagattcatttctcta